European Patent Application EP 4 752 225 A1, published June 3, 2026. Title: Novel plant promoters. Applicant: KWS SAAT SE & Co. KGaA. Application EP. The sequence listing filed with the application follows.

SEQUENCE LISTING (4 sequences)

SEQ ID NO: 1 - DNA, 1233 bp, synthetic construct
  source 1..1233: mol_type = other DNA
caagaaacaaccgcagcgtcagcgagcggccatagaagcatggcgagtatcaagtagcaccttcctgcgaacgtgggggtgtgtggatgggtcgaagagaggagggggcagattgggaatcagggcgggtgcgcagcagggctcgtacacttgagcgaggcggtgtactgggggaagcaggcggagtcggcgatcctggcggcgctggggtacggcggctgcggcggcgacatccctggagacgcgcggtggtgggttggggacgccgacgctgcctgtgccgtcgccatggtgccccgcgtccttttcttcgctagttcggttcttcctccttttcgggctttcgattggccgtcgtctttctggatggggcgaagtgatggacagggctttggtaatgggctgcttatcttccgattactagtactgggccagatggacggagtactgggccaacgaagcgaatgagtacctgtaaagcagataaataacccttctgcatgactgcatctgagatgattgcgcaggtaaactttgcgttggagaagaattacgacgacggagtagatcctgttgtgattgtgagacaagatctcgatttgtattccggccggtggcacttaagaaatgacctcttgacccggcccgatcggatcttgaaaaaaaaagcagcagtttttacgagtttaaaactcagcggggggtggggtggggtggtggaaatggaatctggatggctcacactttaacattagagcaactccatggctaatacaataccaatagttcacacttaacattagagcaactccactatactcggcaaataaataactaaatttattgatttagctactctctaaaataggttttaaaaaaataggttaatcaaatatactctataaaccaatttattagatagtgagtgaagaagactataaaaaaatagaaagcggagacggaggaacgaagagcagttaaaattgaaaaatcatttacagagtttgttggatatttttttcatctaataataactaattttaactttacaaaatgatttgtctaatcttttgaagttgctcgtgaatactacgactaaaacatggtgatgggtaacaccgtagcaggcaatcatatctatatggtaatccgggactcgtcagcagaggcacagctggagcaaagcaaccagagggagcgcgagccggccactcccctccgtctctctcgacc

SEQ ID NO: 2 - DNA, 698 bp, synthetic construct
  source 1..698: mol_type = other DNA
aacgtcgacacatttaatgcttaatctaacaataattacttttatatatttgatcgaactttaaaagatttggctcctcagaaagatagacgatgtgcatttattttagaaatgataggatatatttaaggcgacatatggaatagacaggttgggatggagtagatatatatagattcatacgactaaagttgtgttcagcagatcatatatatagctatgcaaaacactattttacactgtagatagcaatatttatgttgtttagagagtgaattttgaaataagaggtgagatagagaatgtgatatggcagctaagagctagttttcaacaagtttgtttctataatagtatagctagatagacagacacgtagctaaaatggtcaactgaccttcgtacaaaaaaaaactttaatccagagatatagcaatatatgcttataactccagacctcagagtcaacccacagatttttgtatattcgtcaaaaagatccacagatttgtggtagagagtatgttttagtagtagtggtatatctcccttgtgggacgacgaagcagccggtcagccggcgctccggccggccggccggcctgcgcctgcacagtacaaatagcaccccccgtcctccagttggctgcatccttctagcttcgatctctatatacctctgtatgtgagtgaggcca

SEQ ID NO: 3 - DNA, 976 bp, synthetic construct
  source 1..976: mol_type = other DNA
tcaaacaccatcatacattcttccttttatctgtaagacaaaaaaactaaccaaacctcattattttggactgaattaaactgaactataccgaactgagttgaacagaagtaaaatgacatgagaaaagttcataaactaaactaactaaattaaaaggatttttctatgttatacccttgtgttttttcaatttatacgttgtaccccaagcttttaaaaattccacacggcactctcaaacttaccatttttaatgcaccatgcccctatcactgattatacgtcactaatttcgtgtactttttataatatagtggaatgaatctaatttgcaaataatccctctaagagttaaattatgtataagtcaaatcagttccaataaattttaaaaaaggaacgaaattaatgatatataatcagcagtttgggcatcttgtactaaaaaaaggtaaggttgagggtatcgtgtagaatttttaaaaggttgtggtacaacgtagaaactgaagaaacacaaagtatagcgtagaagatcccaaattaaaattatgccaaaaaagagggcctaaccaaacctcattattttggattgaattaaactgaactatatcgaactgagttgaaatgaagtaaaacgatatgagacaagtttataaactaaactaactaaattaaaattatgccaaaaaaaggggcctaacccccttgtagaattttaaattttacatatcctttggcaaaagaatattcgatgcctcattggctcattgttgctcaacacacaagattggtgattagtccatcacattcttgtttcttgacaatcgacttaccactctccttcctacctaaaatctactttacagtttacacagatcatcatcatatcatcttgataatctaaactttgacacccccctaaaattagaccaattccaaaaaaatcccctcatctctgaatcattccacc

SEQ ID NO: 4 - DNA, 1701 bp, synthetic construct
  source 1..1701: mol_type = other DNA
tataagttcaaacttcaatacaggtattttcgggatgtgattaccttacaatttctcattttcaaagaattttacctgtgcagctatgttggataacctgtgcgagattccgtttcagtaggacactttttttttttaccaataaaaaaaaacttataagttcatgagctaatttttatagatagtttaaagtaccgggtggaggatgaatagttgagttttttcttcaaaattagatacttcctccgttttttattagatgttacacttttcaaatcacggactcctaggtaatttttggagaggagagagatagagagaatgaaaaacaaaagggtcccatgtgagtatgtgataggagagagatagagagaatttattacccaaaataaaagtgtaacatctaattcaaaacttcctaaaatagaaagtgtaacatctaaaaaaaacggaggaagtatttgaatttgatatagatattgtgtctttgtgtgtgttgaatttcaattcccagttccctaaaaaaaatttacaattgcaatttcgagattatgatgtaaattaaatttgagagactagaaagtatttggtcaacccaaaaaaaaaatatcaatacttatataaatcaaaaacataatagagaatccaattttactaaaaatattagtaattttgattaaaataatctattaaaatgaactctaaccttcacataatttccacatattattaatcaacaaaataagcatcacaaattattagaataggcgatctaattttaacataaaattagacgaattcaaattgaatttttctaacaagctcattccatttcacgcaacccaaaattatcctagtcagtagtcatccattcttttctcattcctttattcttgattatcgaactacaacagataatttcaaaaaaaaactaaattggtagtcttaactgattaaactacttactaaatggattaaagaatgtcattactgaatagattaaactgattacgaaatagattaacttggtccctaaatagattaaattagttactatattaaaattaggcgatctcttacaaaaccaactgaataagcatagctctgtatattacctagatttcaactaaatcaaaaccccttacagttcaatctagagctgatcattttggctcggcccgtcccatttttgggccgggttttagtcagatttttttggcccgcggtcgggcccggcccgatttttttggctttgggcaagccaaaaacgacttttcagtttattttttggcccgacccgtttttacccgcaaaagcccgctaatttaggtccgcactttgggcacaaaaatttagcccgaacttaaacctggcccgacccatgatcacctctagtttaatccaaactaaaaaactacacaagttagccaaaaattatgtctactttgtacaactttataaaatacacacagtagttgatatcttgatgattaactccttttgaagtttgactacacaccaaccccaaacacacccactttttcccccctcttgtcaccaaccccccctcctctttagccaccaaagtttggttggtgagtcctccataactgctaaattctctcttttttctctctcctaaaaaactaaaacccaccaaaatttcagacatcaaaaaaattacaagtgaaggaaacaata